European Patent Application EP 4 365 297 A1, published May 8, 2024. Title: Schutz gegen verschiedene Pathogene durch Ribonukleinsäuren, die experimentell identifiziert oder generiert wurden und zuverlässig effizient im RNA silencing-Prozess wirken. Applicant: Martin-Luther-Universität Halle-Wittenberg. The sequence listing filed with the application follows.

SEQUENCE LISTING (204 sequences)

SEQ ID NO: 1 - RNA, 21 nt, synthetic construct
  source 1..21: mol_type = other RNA
ttgcacctacgttcaattcca

SEQ ID NO: 2 - RNA, 21 nt, synthetic construct
  source 1..21: mol_type = other RNA
tttgaacgcgctctctcgctg

SEQ ID NO: 3 - RNA, 21 nt, synthetic construct
  source 1..21: mol_type = other RNA
ttgctcagatcgcaaacgttc

SEQ ID NO: 4 - RNA, 21 nt, synthetic construct
  source 1..21: mol_type = other RNA
ttgacatcaaatcctgccatc

SEQ ID NO: 5 - RNA, 21 nt, synthetic construct
  source 1..21: mol_type = other RNA
gtattgccaaaataagtgagt

SEQ ID NO: 6 - RNA, 21 nt, synthetic construct
  source 1..21: mol_type = other RNA
tactcttcttatgatacgtta

SEQ ID NO: 7 - RNA, 21 nt, synthetic construct
  source 1..21: mol_type = other RNA
tcgacaccgtaactgccgttc

SEQ ID NO: 8 - RNA, 21 nt, synthetic construct
  source 1..21: mol_type = other RNA
ttgaaaagagttgtgaattta

SEQ ID NO: 9 - RNA, 21 nt, synthetic construct
  source 1..21: mol_type = other RNA
ttaccggcgaaccaatctgta

SEQ ID NO: 10 - RNA, 21 nt, synthetic construct
  source 1..21: mol_type = other RNA
ttacgtttcttaattgctgta

SEQ ID NO: 11 - RNA, 21 nt, synthetic construct
  source 1..21: mol_type = other RNA
tcagatttttcaaggtaatct

SEQ ID NO: 12 - RNA, 21 nt, synthetic construct
  source 1..21: mol_type = other RNA
ttccgcccattcgttaccggc

SEQ ID NO: 13 - RNA, 21 nt, synthetic construct
  source 1..21: mol_type = other RNA
acatggcggcatgaccctgtc

SEQ ID NO: 14 - RNA, 21 nt, synthetic construct
  source 1..21: mol_type = other RNA
tcagatttttcaaggtaatct

SEQ ID NO: 15 - RNA, 21 nt, synthetic construct
  source 1..21: mol_type = other RNA
agagtaagaacttcgaacaaa

SEQ ID NO: 16 - RNA, 21 nt, synthetic construct
  source 1..21: mol_type = other RNA
atagtctgcactttcgacgaa

SEQ ID NO: 17 - RNA, 21 nt, synthetic construct
  source 1..21: mol_type = other RNA
aaatcagatttagtgtaaata

SEQ ID NO: 18 - RNA, 21 nt, synthetic construct
  source 1..21: mol_type = other RNA
actcagctcccgccacagaaa

SEQ ID NO: 19 - RNA, 21 nt, synthetic construct
  source 1..21: mol_type = other RNA
atggacaacccgttcaccaca

SEQ ID NO: 20 - RNA, 21 nt, synthetic construct
  source 1..21: mol_type = other RNA
aaacctaggagatggtttcaa

SEQ ID NO: 21 - RNA, 21 nt, synthetic construct
  source 1..21: mol_type = other RNA
aatgaagaatctctcagccac

SEQ ID NO: 22 - RNA, 21 nt, synthetic construct
  source 1..21: mol_type = other RNA
aaagcgacaaggagctcatca

SEQ ID NO: 23 - RNA, 21 nt, synthetic construct
  source 1..21: mol_type = other RNA
aatagccgcgaccaggtcttc

SEQ ID NO: 24 - RNA, 21 nt, synthetic construct
  source 1..21: mol_type = other RNA
ataaaagaacatttattaaac

SEQ ID NO: 25 - RNA, 21 nt, synthetic construct
  source 1..21: mol_type = other RNA
atacgcatgggtttgaccatc

SEQ ID NO: 26 - RNA, 21 nt, synthetic construct
  source 1..21: mol_type = other RNA
aaagcaccttccgcccattcg

SEQ ID NO: 27 - RNA, 21 nt, synthetic construct
  source 1..21: mol_type = other RNA
gaattgaacgtaggtgcaatg

SEQ ID NO: 28 - RNA, 21 nt, synthetic construct
  source 1..21: mol_type = other RNA
gcgagagagcgcgttcaaatc

SEQ ID NO: 29 - RNA, 21 nt, synthetic construct
  source 1..21: mol_type = other RNA
acgtttgcgatctgagcaacg

SEQ ID NO: 30 - RNA, 21 nt, synthetic construct
  source 1..21: mol_type = other RNA
tggcaggatttgatgtcaaga

SEQ ID NO: 31 - RNA, 21 nt, synthetic construct
  source 1..21: mol_type = other RNA
tcacttattttggcaatacca

SEQ ID NO: 32 - RNA, 21 nt, synthetic construct
  source 1..21: mol_type = other RNA
acgtatcataagaagagtata

SEQ ID NO: 33 - RNA, 21 nt, synthetic construct
  source 1..21: mol_type = other RNA
acggcagttacggtgtcgaca

SEQ ID NO: 34 - RNA, 21 nt, synthetic construct
  source 1..21: mol_type = other RNA
aattcacaactcttttcaaca

SEQ ID NO: 35 - RNA, 21 nt, synthetic construct
  source 1..21: mol_type = other RNA
cagattggttcgccggtaacg

SEQ ID NO: 36 - RNA, 21 nt, synthetic construct
  source 1..21: mol_type = other RNA
cagcaattaagaaacgtaatg

SEQ ID NO: 37 - RNA, 21 nt, synthetic construct
  source 1..21: mol_type = other RNA
attaccttgaaaaatctgatg

SEQ ID NO: 38 - RNA, 21 nt, synthetic construct
  source 1..21: mol_type = other RNA
cggtaacgaatgggcggaagg

SEQ ID NO: 39 - RNA, 21 nt, synthetic construct
  source 1..21: mol_type = other RNA
cagggtcatgccgccatgtga

SEQ ID NO: 40 - RNA, 21 nt, synthetic construct
  source 1..21: mol_type = other RNA
catgttagacttcgacagtct

SEQ ID NO: 41 - RNA, 21 nt, synthetic construct
  source 1..21: mol_type = other RNA
tgttcgaagttcttactctct

SEQ ID NO: 42 - RNA, 21 nt, synthetic construct
  source 1..21: mol_type = other RNA
cgtcgaaagtgcagactattc

SEQ ID NO: 43 - RNA, 21 nt, synthetic construct
  source 1..21: mol_type = other RNA
tttacactaaatctgatttct

SEQ ID NO: 44 - RNA, 21 nt, synthetic construct
  source 1..21: mol_type = other RNA
tctgtggcgggagctgagttg

SEQ ID NO: 45 - RNA, 21 nt, synthetic construct
  source 1..21: mol_type = other RNA
tggtgaacgggttgtccatcc

SEQ ID NO: 46 - RNA, 21 nt, synthetic construct
  source 1..21: mol_type = other RNA
gaaaccatctcctaggtttct

SEQ ID NO: 47 - RNA, 21 nt, synthetic construct
  source 1..21: mol_type = other RNA
ggctgagagattcttcatttc

SEQ ID NO: 48 - RNA, 21 nt, synthetic construct
  source 1..21: mol_type = other RNA
atgagctccttgtcgcttttg

SEQ ID NO: 49 - RNA, 21 nt, synthetic construct
  source 1..21: mol_type = other RNA
agacctggtcgcggctattta

SEQ ID NO: 50 - RNA, 21 nt, synthetic construct
  source 1..21: mol_type = other RNA
ttaataaatgttcttttattt

SEQ ID NO: 51 - RNA, 21 nt, synthetic construct
  source 1..21: mol_type = other RNA
tggtcaaacccatgcgtatcg

SEQ ID NO: 52 - RNA, 21 nt, synthetic construct
  source 1..21: mol_type = other RNA
aatgggcggaaggtgctttct

SEQ ID NO: 53 - RNA, 21 nt, synthetic construct
  source 1..21: mol_type = other RNA
acacacacacgcacacacaca

SEQ ID NO: 54 - RNA, 21 nt, synthetic construct
  source 1..21: mol_type = other RNA
ttaaagtcctactggtacctt

SEQ ID NO: 55 - RNA, 21 nt, synthetic construct
  source 1..21: mol_type = other RNA
tcacactcagtagccattttc

SEQ ID NO: 56 - RNA, 21 nt, synthetic construct
  source 1..21: mol_type = other RNA
attcaccaacatcatatccag

SEQ ID NO: 57 - RNA, 21 nt, synthetic construct
  source 1..21: mol_type = other RNA
ataactccttgtcgcccagat

SEQ ID NO: 58 - RNA, 21 nt, synthetic construct
  source 1..21: mol_type = other RNA
attgcccatctatgggagata

SEQ ID NO: 59 - RNA, 21 nt, synthetic construct
  source 1..21: mol_type = other RNA
taacgaaacgcattgcccatc

SEQ ID NO: 60 - RNA, 21 nt, synthetic construct
  source 1..21: mol_type = other RNA
aacaccgcttacgattcccaa

SEQ ID NO: 61 - RNA, 21 nt, synthetic construct
  source 1..21: mol_type = other RNA
aaacaccgcttacgattccca

SEQ ID NO: 62 - RNA, 21 nt, synthetic construct
  source 1..21: mol_type = other RNA
aaggcagtactagagtcttcc

SEQ ID NO: 63 - RNA, 21 nt, synthetic construct
  source 1..21: mol_type = other RNA
ttatatactaatacgcaccaa

SEQ ID NO: 64 - RNA, 21 nt, synthetic construct
  source 1..21: mol_type = other RNA
tacttatatactaatacgcac

SEQ ID NO: 65 - RNA, 21 nt, synthetic construct
  source 1..21: mol_type = other RNA
atagatatagtattatgtaca

SEQ ID NO: 66 - RNA, 21 nt, synthetic construct
  source 1..21: mol_type = other RNA
ttactaaaaccagatgtgttc

SEQ ID NO: 67 - RNA, 21 nt, synthetic construct
  source 1..21: mol_type = other RNA
aagaggaattgaacctcaaaa

SEQ ID NO: 68 - RNA, 21 nt, synthetic construct
  source 1..21: mol_type = other RNA
aacgtcttattaagtcgcgaa

SEQ ID NO: 69 - RNA, 21 nt, synthetic construct
  source 1..21: mol_type = other RNA
aacaagcttcttatcatattc

SEQ ID NO: 70 - RNA, 21 nt, synthetic construct
  source 1..21: mol_type = other RNA
ttctccacgactgaccatttt

SEQ ID NO: 71 - RNA, 21 nt, synthetic construct
  source 1..21: mol_type = other RNA
aaggcgcctcagagatttgta

SEQ ID NO: 72 - RNA, 21 nt, synthetic construct
  source 1..21: mol_type = other RNA
taccctgaaactagcacgttg

SEQ ID NO: 73 - RNA, 21 nt, synthetic construct
  source 1..21: mol_type = other RNA
tgtgtgtgcgtgtgtgtgtgt

SEQ ID NO: 74 - RNA, 21 nt, synthetic construct
  source 1..21: mol_type = other RNA
ggtaccagtaggactttaact

SEQ ID NO: 75 - RNA, 21 nt, synthetic construct
  source 1..21: mol_type = other RNA
aaatggctactgagtgtgacc

SEQ ID NO: 76 - RNA, 21 nt, synthetic construct
  source 1..21: mol_type = other RNA
ggatatgatgttggtgaatta

SEQ ID NO: 77 - RNA, 21 nt, synthetic construct
  source 1..21: mol_type = other RNA
ctgggcgacaaggagttatct

SEQ ID NO: 78 - RNA, 21 nt, synthetic construct
  source 1..21: mol_type = other RNA
tctcccatagatgggcaatgc

SEQ ID NO: 79 - RNA, 21 nt, synthetic construct
  source 1..21: mol_type = other RNA
tgggcaatgcgtttcgttaca

SEQ ID NO: 80 - RNA, 21 nt, synthetic construct
  source 1..21: mol_type = other RNA
gggaatcgtaagcggtgtttt

SEQ ID NO: 81 - RNA, 21 nt, synthetic construct
  source 1..21: mol_type = other RNA
ggaatcgtaagcggtgttttg

SEQ ID NO: 82 - RNA, 21 nt, synthetic construct
  source 1..21: mol_type = other RNA
aagactctagtactgcctttc

SEQ ID NO: 83 - RNA, 21 nt, synthetic construct
  source 1..21: mol_type = other RNA
ggtgcgtattagtatataagt

SEQ ID NO: 84 - RNA, 21 nt, synthetic construct
  source 1..21: mol_type = other RNA
gcgtattagtatataagtatt

SEQ ID NO: 85 - RNA, 21 nt, synthetic construct
  source 1..21: mol_type = other RNA
tacataatactatatctatag

SEQ ID NO: 86 - RNA, 21 nt, synthetic construct
  source 1..21: mol_type = other RNA
acacatctggttttagtaagc

SEQ ID NO: 87 - RNA, 21 nt, synthetic construct
  source 1..21: mol_type = other RNA
ttgaggttcaattcctcttac

SEQ ID NO: 88 - RNA, 21 nt, synthetic construct
  source 1..21: mol_type = other RNA
cgcgacttaataagacgttag

SEQ ID NO: 89 - RNA, 21 nt, synthetic construct
  source 1..21: mol_type = other RNA
atatgataagaagcttgtttc

SEQ ID NO: 90 - RNA, 21 nt, synthetic construct
  source 1..21: mol_type = other RNA
aatggtcagtcgtggagaaat

SEQ ID NO: 91 - RNA, 21 nt, synthetic construct
  source 1..21: mol_type = other RNA
caaatctctgaggcgcctttg

SEQ ID NO: 92 - RNA, 21 nt, synthetic construct
  source 1..21: mol_type = other RNA
acgtgctagtttcagggtacg

SEQ ID NO: 93 - RNA, 21 nt, synthetic construct
  source 1..21: mol_type = other RNA
aaagagcagttttgtcaacaa

SEQ ID NO: 94 - RNA, 21 nt, synthetic construct
  source 1..21: mol_type = other RNA
aagcttctctttcccgaattt

SEQ ID NO: 95 - RNA, 21 nt, synthetic construct
  source 1..21: mol_type = other RNA
aaaagcgtttatcgtcgatgg

SEQ ID NO: 96 - RNA, 21 nt, synthetic construct
  source 1..21: mol_type = other RNA
aagctgaggatagcgcttgta

SEQ ID NO: 97 - RNA, 21 nt, synthetic construct
  source 1..21: mol_type = other RNA
atatttctcttcttggccttc

SEQ ID NO: 98 - RNA, 21 nt, synthetic construct
  source 1..21: mol_type = other RNA
atgggccgatggagtggagca

SEQ ID NO: 99 - RNA, 21 nt, synthetic construct
  source 1..21: mol_type = other RNA
atttcgaaaatgtccacgtct

SEQ ID NO: 100 - RNA, 21 nt, synthetic construct
  source 1..21: mol_type = other RNA
aatccttttgacccattccaa

SEQ ID NO: 101 - RNA, 21 nt, synthetic construct
  source 1..21: mol_type = other RNA
aaagtcaagatacctcttttg

SEQ ID NO: 102 - RNA, 21 nt, synthetic construct
  source 1..21: mol_type = other RNA
atgttcttcaggagcaacacg

SEQ ID NO: 103 - RNA, 21 nt, synthetic construct
  source 1..21: mol_type = other RNA
agaacggcttggatggcaaca

SEQ ID NO: 104 - RNA, 21 nt, synthetic construct
  source 1..21: mol_type = other RNA
aagcatacaaagaaagaacgg

SEQ ID NO: 105 - RNA, 21 nt, synthetic construct
  source 1..21: mol_type = other RNA
agaagcatacaaagaaagaac

SEQ ID NO: 106 - RNA, 21 nt, synthetic construct
  source 1..21: mol_type = other RNA
aagcaacatagcaaagcttct

SEQ ID NO: 107 - RNA, 21 nt, synthetic construct
  source 1..21: mol_type = other RNA
gttgacaaaactgctcttttc

SEQ ID NO: 108 - RNA, 21 nt, synthetic construct
  source 1..21: mol_type = other RNA
attcgggaaagagaagcttca

SEQ ID NO: 109 - RNA, 21 nt, synthetic construct
  source 1..21: mol_type = other RNA
atcgacgataaacgcttttga

SEQ ID NO: 110 - RNA, 21 nt, synthetic construct
  source 1..21: mol_type = other RNA
caagcgctatcctcagctttg

SEQ ID NO: 111 - RNA, 21 nt, synthetic construct
  source 1..21: mol_type = other RNA
aggccaagaagagaaatatcg

SEQ ID NO: 112 - RNA, 21 nt, synthetic construct
  source 1..21: mol_type = other RNA
ctccactccatcggcccatag

SEQ ID NO: 113 - RNA, 21 nt, synthetic construct
  source 1..21: mol_type = other RNA
acgtggacattttcgaaatcg

SEQ ID NO: 114 - RNA, 21 nt, synthetic construct
  source 1..21: mol_type = other RNA
ggaatgggtcaaaaggattcg

SEQ ID NO: 115 - RNA, 21 nt, synthetic construct
  source 1..21: mol_type = other RNA
aaagaggtatcttgactttga

SEQ ID NO: 116 - RNA, 21 nt, synthetic construct
  source 1..21: mol_type = other RNA
tgttgctcctgaagaacatcc

SEQ ID NO: 117 - RNA, 21 nt, synthetic construct
  source 1..21: mol_type = other RNA
ttgccatccaagccgttcttt

SEQ ID NO: 118 - RNA, 21 nt, synthetic construct
  source 1..21: mol_type = other RNA
gttctttctttgtatgcttct

SEQ ID NO: 119 - RNA, 21 nt, synthetic construct
  source 1..21: mol_type = other RNA
tctttctttgtatgcttctgg

SEQ ID NO: 120 - RNA, 21 nt, synthetic construct
  source 1..21: mol_type = other RNA
aagctttgctatgttgctttg

SEQ ID NO: 121 - RNA, 21 nt, synthetic construct
  source 1..21: mol_type = other RNA
ccctccaactcgcgctccatt

SEQ ID NO: 122 - RNA, 21 nt, synthetic construct
  source 1..21: mol_type = other RNA
taacacttcctcttcgcaatc

SEQ ID NO: 123 - RNA, 21 nt, synthetic construct
  source 1..21: mol_type = other RNA
taagggaagcgagtgagactt

SEQ ID NO: 124 - RNA, 21 nt, synthetic construct
  source 1..21: mol_type = other RNA
ttgtcgcaagtgaattcgagg

SEQ ID NO: 125 - RNA, 21 nt, synthetic construct
  source 1..21: mol_type = other RNA
ttgcttgcatccgggattgtc

SEQ ID NO: 126 - RNA, 21 nt, synthetic construct
  source 1..21: mol_type = other RNA
tatctcttgcttgcatccggg

SEQ ID NO: 127 - RNA, 21 nt, synthetic construct
  source 1..21: mol_type = other RNA
ctcatcaaagactgtagaaag

SEQ ID NO: 128 - RNA, 21 nt, synthetic construct
  source 1..21: mol_type = other RNA
tatcctcatcaaagactgtag

SEQ ID NO: 129 - RNA, 21 nt, synthetic construct
  source 1..21: mol_type = other RNA
tttgacgataccatacatgtt

SEQ ID NO: 130 - RNA, 21 nt, synthetic construct
  source 1..21: mol_type = other RNA
tttcacttaattctaccccag

SEQ ID NO: 131 - RNA, 21 nt, synthetic construct
  source 1..21: mol_type = other RNA
tttttccctttcgaagcaaac

SEQ ID NO: 132 - RNA, 21 nt, synthetic construct
  source 1..21: mol_type = other RNA
tatcaggaaggagcttttgga

SEQ ID NO: 133 - RNA, 21 nt, synthetic construct
  source 1..21: mol_type = other RNA
tatttgtgcgacttgctctct

SEQ ID NO: 134 - RNA, 21 nt, synthetic construct
  source 1..21: mol_type = other RNA
taataacatatataggtttcc

SEQ ID NO: 135 - RNA, 21 nt, synthetic construct
  source 1..21: mol_type = other RNA
tttcgtactatcaatcgagat

SEQ ID NO: 136 - RNA, 21 nt, synthetic construct
  source 1..21: mol_type = other RNA
taaccccgctttcgtactatc

SEQ ID NO: 137 - RNA, 21 nt, synthetic construct
  source 1..21: mol_type = other RNA
ttactcttcaataaccccgct

SEQ ID NO: 138 - RNA, 21 nt, synthetic construct
  source 1..21: mol_type = other RNA
ttcttttgtgtgcttctactg

SEQ ID NO: 139 - RNA, 21 nt, synthetic construct
  source 1..21: mol_type = other RNA
tatccccccttcttcgagatc

SEQ ID NO: 140 - RNA, 21 nt, synthetic construct
  source 1..21: mol_type = other RNA
tatcagattttccttcagtga

SEQ ID NO: 141 - RNA, 21 nt, synthetic construct
  source 1..21: mol_type = other RNA
tttcgctcgatgtgaagttgc

SEQ ID NO: 142 - RNA, 21 nt, synthetic construct
  source 1..21: mol_type = other RNA
tttccctgagacttagctttc

SEQ ID NO: 143 - RNA, 21 nt, synthetic construct
  source 1..21: mol_type = other RNA
tatcctgccatctatatacat

SEQ ID NO: 144 - RNA, 21 nt, synthetic construct
  source 1..21: mol_type = other RNA
ttcaaccccaagaaaatgaac

SEQ ID NO: 145 - RNA, 21 nt, synthetic construct
  source 1..21: mol_type = other RNA
tatacacttttcaagtcgcac

SEQ ID NO: 146 - RNA, 21 nt, synthetic construct
  source 1..21: mol_type = other RNA
tatcggtgagagcatatacac

SEQ ID NO: 147 - RNA, 21 nt, synthetic construct
  source 1..21: mol_type = other RNA
taacatctgcggaataagtgg

SEQ ID NO: 148 - RNA, 21 nt, synthetic construct
  source 1..21: mol_type = other RNA
tatccctgcattcaagactac

SEQ ID NO: 149 - RNA, 21 nt, synthetic construct
  source 1..21: mol_type = other RNA
ttgcgcagcttcatcgtcgga

SEQ ID NO: 150 - RNA, 21 nt, synthetic construct
  source 1..21: mol_type = other RNA
ttcctcagctgatcgagggta

SEQ ID NO: 151 - RNA, 21 nt, synthetic construct
  source 1..21: mol_type = other RNA
tggagcgcgagttggagggat

SEQ ID NO: 152 - RNA, 21 nt, synthetic construct
  source 1..21: mol_type = other RNA
ttgcgaagaggaagtgttagc

SEQ ID NO: 153 - RNA, 21 nt, synthetic construct
  source 1..21: mol_type = other RNA
gtctcactcgcttcccttacc

SEQ ID NO: 154 - RNA, 21 nt, synthetic construct
  source 1..21: mol_type = other RNA
tcgaattcacttgcgacaatc

SEQ ID NO: 155 - RNA, 21 nt, synthetic construct
  source 1..21: mol_type = other RNA
caatcccggatgcaagcaaga

SEQ ID NO: 156 - RNA, 21 nt, synthetic construct
  source 1..21: mol_type = other RNA
cggatgcaagcaagagatacc

SEQ ID NO: 157 - RNA, 21 nt, synthetic construct
  source 1..21: mol_type = other RNA
ttctacagtctttgatgagga

SEQ ID NO: 158 - RNA, 21 nt, synthetic construct
  source 1..21: mol_type = other RNA
acagtctttgatgaggatatg

SEQ ID NO: 159 - RNA, 21 nt, synthetic construct
  source 1..21: mol_type = other RNA
catgtatggtatcgtcaaatt

SEQ ID NO: 160 - RNA, 21 nt, synthetic construct
  source 1..21: mol_type = other RNA
ggggtagaattaagtgaaacg

SEQ ID NO: 161 - RNA, 21 nt, synthetic construct
  source 1..21: mol_type = other RNA
ttgcttcgaaagggaaaaaca

SEQ ID NO: 162 - RNA, 21 nt, synthetic construct
  source 1..21: mol_type = other RNA
caaaagctccttcctgatatc

SEQ ID NO: 163 - RNA, 21 nt, synthetic construct
  source 1..21: mol_type = other RNA
agagcaagtcgcacaaataca

SEQ ID NO: 164 - RNA, 21 nt, synthetic construct
  source 1..21: mol_type = other RNA
aaacctatatatgttattact

SEQ ID NO: 165 - RNA, 21 nt, synthetic construct
  source 1..21: mol_type = other RNA
ctcgattgatagtacgaaagc

SEQ ID NO: 166 - RNA, 21 nt, synthetic construct
  source 1..21: mol_type = other RNA
tagtacgaaagcggggttatt

SEQ ID NO: 167 - RNA, 21 nt, synthetic construct
  source 1..21: mol_type = other RNA
cggggttattgaagagtaata

SEQ ID NO: 168 - RNA, 21 nt, synthetic construct
  source 1..21: mol_type = other RNA
gtagaagcacacaaaagaacg

SEQ ID NO: 169 - RNA, 21 nt, synthetic construct
  source 1..21: mol_type = other RNA
tctcgaagaaggggggatatg

SEQ ID NO: 170 - RNA, 21 nt, synthetic construct
  source 1..21: mol_type = other RNA
actgaaggaaaatctgatatc

SEQ ID NO: 171 - RNA, 21 nt, synthetic construct
  source 1..21: mol_type = other RNA
aacttcacatcgagcgaaagc

SEQ ID NO: 172 - RNA, 21 nt, synthetic construct
  source 1..21: mol_type = other RNA
aagctaagtctcagggaaatg

SEQ ID NO: 173 - RNA, 21 nt, synthetic construct
  source 1..21: mol_type = other RNA
gtatatagatggcaggatacg

SEQ ID NO: 174 - RNA, 21 nt, synthetic construct
  source 1..21: mol_type = other RNA
tcattttcttggggttgaagt

SEQ ID NO: 175 - RNA, 21 nt, synthetic construct
  source 1..21: mol_type = other RNA
gcgacttgaaaagtgtatatg

SEQ ID NO: 176 - RNA, 21 nt, synthetic construct
  source 1..21: mol_type = other RNA
gtatatgctctcaccgatagg

SEQ ID NO: 177 - RNA, 21 nt, synthetic construct
  source 1..21: mol_type = other RNA
acttattccgcagatgttaaa

SEQ ID NO: 178 - RNA, 21 nt, synthetic construct
  source 1..21: mol_type = other RNA
agtcttgaatgcagggatagg

SEQ ID NO: 179 - RNA, 21 nt, synthetic construct
  source 1..21: mol_type = other RNA
cgacgatgaagctgcgcaacc

SEQ ID NO: 180 - RNA, 21 nt, synthetic construct
  source 1..21: mol_type = other RNA
ccctcgatcagctgaggaaag

SEQ ID NO: 181 - RNA, 170 nt, synthetic construct
  source 1..170: mol_type = other RNA
gggcgaattgggtaccgggcattacgtttcttaattgctgtatactcttcttatgatacgttatcagatttttcaaggtaatcttgatgagctccttgtcgcttttttgttcgaagttcttactctttcgtcgaaagtgcagactattctcagatctgccggtctcccta

SEQ ID NO: 182 - RNA, 178 nt, synthetic construct
  source 1..178: mol_type = other RNA
gggcgaattgggtaccgggccattacgtttcttaattgctgtaatactcttcttatgatacgttattcagatttttcaaggtaatcttatgatgagctccttgtcgctttatttgttcgaagttcttactctgttcgtcgaaagtgcagactattcatcagatctgccggtctcccta

SEQ ID NO: 183 - RNA, 170 nt, synthetic construct
  source 1..170: mol_type = other RNA
gggcgaattgggtaccggggaataaccgggtacatcgcgagacgagatatctatctgagcgtcgtcggcttcacactcttcactgtagtagaaatcagatttagtgtaaatagccgcgaccaggtcttcaaaacacttcatggttcggttcagatctgccggtctcccta

SEQ ID NO: 184 - RNA, 170 nt, synthetic construct
  source 1..170: mol_type = other RNA
gggcgaattgggtaccgggcaagatctgagtccggacttgtatagttcatccatgccatgtgtaatcccagcagctgttacaaactcaagaaggaccatgtggtctctcttttcgttgggatctttcgaaagggcagattgtgtggacatcagatctgccggtctcccta

SEQ ID NO: 185 - RNA, 170 nt, synthetic construct
  source 1..170: mol_type = other RNA
atcccgcttaacccatggcccgtaatgcaaagaattaacgacatatgagaagaatactatgcaatagtctaaaaagttccattagaactactcgaggaacagcgaaaaaacaagcttcaagaatgagaaagcagctttcacgtctgataagagtctagacggccagaggg

SEQ ID NO: 186 - RNA, 178 nt, synthetic construct
  source 1..178: mol_type = other RNA
atcccgcttaacccatggcccggtaatgcaaagaattaacgacattatgagaagaatactatgcaataagtctaaaaagttccattagaatactactcgaggaacagcgaaataaacaagcttcaagaatgagacaagcagctttcacgtctgataagtagtctagacggccagaggg

SEQ ID NO: 187 - RNA, 170 nt, synthetic construct
  source 1..170: mol_type = other RNA
atcccgcttaacccatggccccttattggcccatgtagcgctctgctctatagatagactcgcagcagccgaagtgtgagaagtgacatcatctttagtctaaatcacatttatcggcgctggtccagaagttttgtgaagtaccaagccaagtctagacggccagaggg

SEQ ID NO: 188 - RNA, 170 nt, synthetic construct
  source 1..170: mol_type = other RNA
atcccgcttaacccatggcccgttctagactcaggcctgaacatatcaagtaggtacggtacacattagggtcgtcgacaatgtttgagttcttcctggtacaccagagagaaaagcaaccctagaaagctttcccgtctaacacacctgtagtctagacggccagaggg

SEQ ID NO: 189 - RNA, 3050 nt, Cucumber mosaic virus
  source 1..3050: mol_type = transcribed RNA
gtttatttacaagagcgtacggttcaacccctgcctcccctgtaaaactccctagacttaaatcttttctttctagtatcttttctatggctttccctgcccccgcattctcactagccaatcttttgaacggcagttacggtgtcgacactcccgaggatgtggaacgtttgcgatctgagcaacgcgaagaggctgctgcggcctgtcgtaattacaggcccctacccgctgtggatgtcagcgagagtgtcacagaggacgcgcattccctccgaactcctgacggagctcccgctgaagcggtgtctgatgagtttgtaacttatggtgctgaagattaccttgaaaaatctgatgatgagctccttgtcgcttttgagacgatggtcaaacccatgcgtatcggacaactatggtgccctgcgtttaataaatgttcttttatttccagcattgctatggccagagctttgttgttggcacctagaacatcccaccgaaccatgaagtgttttgaagacctggtcgcggctatttacactaaatctgatttctactacagtgaagagtgtgaagccgacgacgctcagatagatatctcgtctcgcgatgtacccggttattctttcgaaccgtggtcccgaacgtctggatttgaaccgccgcccatttgtgaagcgtgcgacatgatcatgtaccagtgcccgtgttttgattttaatgctttaaagaaatcgtgcgctgagaggaccttcgctgatgattatgttattgaaggtttagatggtgttgttgataatgcgactctgttgtcgaatttgggtccatttttggtacccgtgaagtgtcaatatgaaaaatgtccaacgccaaccatcgcgattcctccggatttaaaccgtgctactgatcgtgttgatatcaatttagttcaatccatttgtgactcgactctgcccactcatagtaattacgacgactcttttcatcaagtgttcgtcgaaagtgcagactattctatagatctggatcatgttagacttcgacagtctgatcttattgcaaaaattccagattcagggcatatgataccggttctgaacaccgggagcggtcacaagagagtaggtacaacgaaggaggtccttacagcaattaagaaacgtaatgctgacgttccagagctaggtgattccgttaatttgtctagattgagtaaagctgtggctgagagattcttcatttcatacatcaatggtaactctctagcatccagtaactttgtcaatgtcgttagtaacttccacgattacatggaaaaatggaagtcctcaggtctttcttatgatgatcttccggatcttcatgctgagaatttgcagttttatgaccacatgataaaatccgatgtgaaacctgtggtgagcgacacactcaatatcgacagaccggttccagctactataacgtatcataagaagagtataacctcccagttctcaccgttattcacagcgctattcgagcgcttccagagatgccttcgagaacgtattattcttcctgttggtaagatttcatcccttgagatggcaggatttgatgtcaagaacaagcactgcctcgagattgacctgtctaagtttgataagtctcaaggtgaatttcacttgctaatccaggaacacattttgaatggtctaggatgtccagctccgataactaagtggtggtgtgatttccatcgattctcttacattagagaccgtagagctggtgttggtatgcctattagtttccagagacgaactggcgatgcactcacttattttggcaataccatcgtcaccatggctgagtttgcctggtgttatgacaccgaccaattcgaaaagcttttattctcaggcgatgattctctaggattttcactgcttccccctgttggtgacccgagtaaattcacaactcttttcaacatggaagctaaggtgatggaacctgccgtaccatatatttgttcgaagttcttactctctgacgagttcggtaacacattttccgttccagatccattgcgcgaggttcagcggttaggaacaaagaaaattccctattctgacaatgatgaattcttgtttgctcacttcatgagctttgttgatcgattgaagtttttggaccgaatgtctcagtcgtgtatcgatcaactttcgattttcttcgaattgaaatacaagaagtctggggaagaggctgctttaatgttaggcgcctttaagaagtataccgctaatttccagtcctacaaagaactctattattcagatcgtcgtcagtgcgaattgatcaattcgttttgtagtacagagttcagggttgagcgtgtaaattccaacaaacagcgaaagaattatggaattgaacgtaggtgcaatgacaaacgtcgaactccaactggctcgtatggtggaggcgaagaagcagagacgaaggtctcacaaacagaatcgacgggaacgaggtcacaaaagtcccagcgagagagcgcgttcaaatctcagactattccgcttcctaccgttctatcaagtggatggttcggaactgacagggtcatgccgccatgtgaacgtggcggagttacccgagtctgaggcctctcgtttagagttatcggcggaagaccatgattttgacgatacagattggttcgccggtaacgaatgggcggaaggtgctttctgaaacctccccttccgcatctccctccggttttctgtggcgggagctgagttggcagtattgctataaactgtctgaagtcactaaacacattgtggtgaacgggttgtccatccagcttacggctaaaatggtcagtcgtagaggaatctacgccagcagacttacaagtctctgaggcacctttgaaaccatctcctaggtttcttcggaaggacttcggtccgtgtacttctagcacaacgtgctagtttcagggtacgggtgccccccacttttgtggggcctccaaaaggagacca

SEQ ID NO: 190 - RNA, 2216 nt, Cucumber mosaic virus
  source 1..2216: mol_type = transcribed RNA
gtaatcttaccactgtgtgtgtgcgtgtgtgtgtgtcgagtcgtgttgtccgcacatttgagtcgtgctgtccgcacatattttatcttttgggtacagtgtgttagatttcccgaggcatggctttccaaggtaccagtaggactttaactcaacagtcctcagcggctacgtctgacgatcttcaaaagatattatttagccctgaagccattaagaaaatggctactgagtgtgacctaggccggcatcattggatgcgcgctgataatgctatttcagtccggcccctcgttcccgaagtaacccacggtcgtattgcttccttctttaagtctggatatgatgttggtgaattatgctcaaaaggatacatgagtgtccctcaagtgttatgtgctgttactcgaacagtttccactgatgctgaagggtctttgagaatttacttagctgatctgggcgacaaggagttatctcccatagatgggcaatgcgtttcgttacataaccatgatcttcccgctttggtgtctttccaaccgacgtatgattgtcctatggaaacagttgggaatcgtaagcggtgttttgctgtcgttatcgaaagacatggttacattgggtataccggtaccacagctagcgtgtgtagtaattggcaagcaaggttttcatccaagaataacaactacactcatatcgcagctgggaagactctagtactgcctttcaacagattagctgagcaaacaaaaccgtcagctgtcgctcgcctgttgaagtcgcaattgaacaacattgaatcttcgcaatatttgttaacgaatgcgaagattaatcaaaatgcgcgcagtgagtccgaggatttaaatgttgagagccctcccgccgcaatcgggagttcttccgcgtcccgctccgaagccttcagaccgcaggtggttaacggtctttagcactttggtgcgtattagtatataagtatttgtgagtctgtacataatactatatctatagtgtcctgtgtgagttgatacagtagacatctgtgacgcgatgccgtgttgagaagggaacacatctggttttagtaagcctacatcatagttttgaggttcaattcctcttactccctgttgagccccttactttctcatggatgcttctccgcgagattgcgttattgtctactgactatatagagagtgtttgtgctgtgttttctcttttgtgtcgtagaattgagtcgagtcatggacaaatctgaatcaaccagtgctggtcgtaaccgtcgacgtcgtccgcgtcgtggttcccgctccgccccctcctccgcggatgctaactttagagtcttgtcgcagcagctttcgcgacttaataagacgttagcagctggtcgtccaactattaaccacccaacctttgtagggagtgaacgctgtagacctgggtacacgttcacatctattaccctaaagccaccaaaaatagaccgtgggtcttattacggtaaaaggttgttactacctgattcagtcacggaatatgataagaagcttgtttcgcgcattcaaattcgagttaatcctttgccgaaatttgattctaccgtgtgggtgacagtccgtaaagttcctgcctcctcggacttatccgttgccgccatctctgctatgttcgcggacggagcctcaccggtactggtttatcagtatgccgcatctggagtccaagccaacaacaaactgttgtatgatctttcggcgatgcgcgctgatataggtgacatgagaaagtacgccgtcctcgtgtattcaaaagacgatgcgctcgagacggacgagctagtacttcatgttgacatcgagcaccaacgcattcccacatctggagtgctcccagtctgattccgtgttcccagaatcctccctccgatctctgtggcgggacgtgagttggcagttctgctataaactgtctgaagtcactaaacgttttttacggtgaacgggttgtccatccagcttacggctaaaatggtcagtcgtggagaaatccacgccagcagatttacaaatctctgaggcgcctttgaaaccatctcctaggtttcttcggaaggacttcggtccgtgtacctctagcacaacgtgctagtttcagggtacgggtgcccccccactttcgtgggggcctccaaaaggagacca

SEQ ID NO: 191 - RNA, 2259 nt, Meloidogyne incognita
  source 1..2259: mol_type = transcribed RNA
atgcctccaatagaaattttggtgcaggctccacaacagcctataaaggtttctggacgtgaggaagattcaatgaataaagaaccctcaatgagtggtcaacaaattgttggtttaattattccacctcctgatattcgaacaattgttgacaaaactgctcttttcgttgcacgtaatggtgttgaatttgaaaataaaattcgggaaagagaagcttcaaatatacgttttaattttcttacacctgtcgacccgtaccatgcttattacaaaaataaagtgaaggaattcgagactggagttgcttctgctgaattattaactaaacttaaaattcctgatgctgttcgtgaacatatacaaaaggctgaatttgttccaaaaaatccgccaaaaccttttgaattttgtgctgatccatcgacgataaacgcttttgatttagatcttatccaacttaccgctctatttgttgcaagaaatggacgtcaatttctcacacaattaatgaatcgagaggtccgcaattttcaattcgactttttaaaacctcaacattccaattttcaatattttacaaaattagtggaacaatacactaaggtgataattccacccaggaatgtgtacgatgaactacgcaattctgcttcacacaaaaaaattttggaagacgttcggtatcgtgttggttgggaaaaatttcaacgtgcagttaaggacagagaagatgctgaagttgaacaagaaaggatggcttataatcaaattgattggcatgattttgtagttgttcaaactgttgattttcaaccttctgaaaccttgaatttaccttcactttgtactcctcgagatgttggagctcgaattttacttcaacaacgaactgaagcagctaaagctgcagctgaaagtgttgcaatggatatggatgaatcagattctgaagatgaagaagagaaaaagaaacagaaaaatagggaagattttgatgatatacaacatcaagtcgatgggatggatattactgaaaaacaacatgctggctctactgttactcagccaacaccagctgcacctattgctgggaatgttgtaatccgtgattatgatcctaaaaaggctcgttccggcatagtggccaaaggacaaaatgaaaaattcatcatttcacctttaacaaatgaacgcattcctgctgataagcttcatgaacacgttcgatacaatactgttgaccctcaatttaaggaacagagagacagggagcaaatggaacgacaagatgaggatccgatcacagcatctggcacggaaatctcacgaaacattgcaaaattagcagagcgacgtactgatattttcggtattggagaaaagggagtagaacaaacaataattggaaagaaattgggtgaagaagagcgtcaattgcctcgttctgaccccaaaacaatctgggatggccaacaagctacaatcgatgccacaacgcgagcggctcaacaagctgtctcccttgaacaacaaataacagaaattcaacgtcaacatggttatttaccaaatccagctgctgatcgttttgcgccaagtacaccgagtacaactgcatcagcgacaacagcttcgaccactactccaatgccaccaccagcaacaacatctgtgccgactccacttccacctcgccctccacacttgcaaccaccaattgtctcaaatgttgccaaaattatacctggcattccaccacaacaacaaatgcgcatgccacgtatgccattacctgggatgcctccacacatgcttccaatgggcatgcaaatgcccggacttcctccacacatggcaatggcccatcacccgcaagcagggtttatgcctccaccacccccacctgatgaaagtggagcttccgctgcaaagaaattccgcgtagatgatgctttggaaccagaagagctttggcttcaaaaagtgtccggccaaataactgtaaagttgagcacaccacatacagatgaatggaatcttaaaggacaaacatttacaatacaattggagattacttcgactgtaagcgcactcaaatcgctaattcaagaacaaacgactgttcccgcatcgaaggccaagcttgtctatcagaatacgtttctcaaagataattttactttggcctattataattttgtgaatgaagcaaatgttcagttaatgttgaaagagcgtggtgggaagaaaaaatag

SEQ ID NO: 192 - RNA, 1128 nt, Meloidogyne incognita
  source 1..1128: mol_type = transcribed RNA
atgtcaaaggcaacgtatggaccaaaacccgagtcttttgtgttggacgatgggcagcggtattatgttggtgctgatgttggaatgtacctcaaatatcatcgtggaaccctttacaagcgctatcctcagctttggaaaagaatggcctctgtagatgaaaagaagaaaattcaagaattgggatgcgcgacttcctatattaattctaatattatgctggtcaaagctagtgaagtagaagaaatctttgaaggccaagaagagaaatatcgctctggaggtgttggctctggaaattatagccgttcagatgccgcaaatattaaaaatcgtggaggtccaaccccttggcttacacaacaggtcaccagtggttctcatcatctcgaatctgtcccttgctccactccatcggcccatagacgtggacattttcgaaatcgcgattatgcttatgctgccgatgacttggaaaattataaacgtgttttgcaaaatgcagagactgctgaatccttggttccgattaggcttgatatggagttggacaatattaaacttcgtgactatttttgctacaacaaaaacgacaaattaatgacccctgaaatgattgctgaagttctttgtgaagacttggatttgcccttaaacacatttttgcctgcaattgcccaatctatacatcaacaaattgaagcacattctgaagctgtacctgtagatgaacaaactactgatcaacgagctcttttaaaattgaatatacatgttgggaatcaatctctagtagatcaatttgaatgggatatgagcgatccaaaaaatagtcctgaagaatttgggcaaaaattgtctgcagaattgggtttgggtggagaatttgttgctgctatagcttattctattagaggtcaattatcctggaatcaacgtacttatgcatttagtgaatctccattaccaaccgtagaatgtccatttcgtaatcctagcgatgcagaacaatgggggccatttttggaaactttaactagcgcagaaattgaaaagaaaatgcgtgatcaggacagaaatactcgaagaatgcgtcgtttagttaatgcaattccttatattccttga

SEQ ID NO: 193 - RNA, 1128 nt, Meloidogyne incognita
  source 1..1128: mol_type = transcribed RNA
atggacgaagaagtagctgctcttgttgttgataatggctcaggcatgtgcaaggctggatttgcgggtgatgatgctcctcgtgccgtttttccaagtattgtcggtcgtcctcgacatcaaggagttatggttggaatgggtcaaaaggattcgtatgtgggagatgaagctcaaagcaaaagaggtatcttgactttgaaatacccgattgagcacggaattgtaacaaactgggacgacatggagaagatttggcatcatacgttctacaatgagttgcgtgttgctcctgaagaacatccagttctccttacagaggcacctctcaacccaaaggctaaccgtgaaaagatgactcaaatcatgtttgagacattcaacacgcctgccatgtatgttgccatccaagccgttctttctttgtatgcttctggacgtactactggaattgttcttgactctggagatggtgttacgcacacagttccaatttatgaaggttatgctttgccacacgcaatcttgcgtcttgacttggcaggacgtgatttgaccgactacttgatgaagatcctcactgaacgtggttattctttcaccacaaccgccgaacgtgagattgtccgtgacatcaaggagaagctttgctatgttgctttggactttgagcaagagatggctacagctgcttcgtcttcttctttggaaaagagctatgaattgcctgacggtcaagtcatcactgttggaaacgagcgcttccgttgcccagaatctctcttccagccatctttcttggggatggaatctgctggtattcatgagacttcttacaactcgatcatgaagtgcgacattgacatccgtaaagacctttacgccaacactgtcctttctggaggtacaaccatgtatccaggcattgctgatcgtatgcagaaggaaattactgctttggcaccatcaacaatgaagattaagattattgcacctcctgagcgtaaatactctgtttggattggaggatctatccttgcttcattgtctaccttccagcaaatgtggatcagcaagcaagagtatgacgaatctggtccatctattgttcaccgtaaatgcttctaa

SEQ ID NO: 194 - RNA, 516 nt, Botrytis cinerea betaendornavirus 1
  source 1..516: mol_type = transcribed RNA
ttcgttccaggagttacacgcaaagatcacttcactggtggaccagcaaaaagatagtaaacatatcgggaaaatatcgatatatattctccgaattctacgagatatcagagcagaattacctagtaaccctgcactacaaaagtttggactctcacttgtctcatcattcgtgctctcgtcgaaagcaaagacaataaagaagaacaaatggagcgcgagttggagggattgcgaagaggaagtgttagcaatcctactacgcatcgtactagtgccatgagcagcggaactgtgactcaggataggaattctctccaagacaataagagcacagttgtaagctggacgttgttcaaagtgcagtggcaaagcgagcacttgaaatgcagttaaagaatgagggactagatgtcactctacaaattgatcaaactcaacaatggttcaatactttgtgggccgacaatggtgacgccatttctaagcaatacgcttctacagcagcattgaagg

SEQ ID NO: 195 - RNA, 2628 nt, Botrytis cinerea betaendornavirus 1
  source 1..2628: mol_type = transcribed RNA
atgtctaccacaagaatctcaacaccgaaaaggtcccccaaaaaatcgacttttgtcaaaactggaatcttgaccaccaaatcaacgcccaatctcaacgcctcctataatttggcattactacaagcttcaggagctacacccgttcctgcatatccttccaataacggtcaaagttttgccctaaataatcctaggtcgcaaccgtctcgacaagtctcactcgcttcccttacctcgaattcacttgcgacaatcccggatgcaagcaagagataccctctttctacagtctttgatgaggatatgccaacagtaggcaacatgccgccatacacacctgctcgagttggcggtggaccggaagaactagaggttggtgatatagtcgatgtgccaggtaacatgtatggtatcgtcaaatttgttggcagtgtgcaaggcaaaaagggtgtatttgctggggtagaattaagtgaaacgtttgcttcgaaagggaaaaacaatggcgatgtcgaaggaattcaatactttgacacaaccatcgatggtgctgggatttttcttccagtcaacagggcgaagagacgtagcaccccttcgtcgcatgatgagtcatttcccctttcaccggcgtctccatcgatgggcaatagggctgggagattaggatctgaattaaatggtcagccaacacctttgttaccaaaattcggtcaatctgttggtccaggcagagcggcaaacccatatgtccaaaaaacacgtccatccatggctacacctaccacctcaagaccggaatcaccagttcgaagagcagccaatgccaacccatcattaaatacacctgcacaaagagtcccatctcgatatgcaagccctgcgcaggcaaactttggacagagcgttagaggaacacaagattctagagatccaagtaagaaagttggctacaccccccgaaatggcatgaaaacaccaatacctccacgaagtgtttctgcacttggaacggggaatagacctgcaccaatgaactcgatgaatttcagtgatgaagagacacctcctgcagagattgcacgtacggcaacaaacggaagcgtaggctcagtctcttctttcaacgcgaaattacgtccagcatcaagatccgcatcgcgtacaacttccagggctaccgacgacgaatttgagcgattgagaagtttgttagaagatcgcgatagggaaataaaagaacaggcttctattatagaagacatggagaaaactctcagtgaagcacaatcgttgatggagaacaataacgagaacgcaagtggtagacatagtcagggaagtgtggatgacaaggacgcaacacagttgagagcaataatacgtgaaaagaacgacaaaatcgccatgctgactgccgagtttgatcagcatcgagctgatttcagaagcacgatagacacgctcgaaatggccggtgcggaaaccgagcgagtgtacgacgagcgcatgcgtgttctcgtaatggagctcgatacaatgcacgagaatagtcatgatgtaaagcacgttgctgtacaactgaaacagctagaagagctcgttcaggagctcgaggaaggtcttgaagatgcacgacgtggtgaagccgaagctcggggagaagttgagttcttgcgtggagaggttgaaagaactcgatctgaactccgccgcgagcgagagaagactgccgaagctcttagcaacgcaaattctcctacgagcgcaagtgcggaaacacattccaaagagattgctcagagagatgacgagattcgtggattgaaagccatcatccactcgctcagcagagatgccatacctgatgggaatttctcggatcatgaggcaacaccaaatattctacgacctggactaaaccgaagtcgaacagaaagtgcttcggtttctgaggaggagcgccgtactcgggaaaagctagagcgagaagtgagtgagcttcgtgctctcgtcgaaagcaaagacaataaagaagaacaaatggagcgcgagttggagggattgcgaagaggaagtgttagcaatcctactacgcatcgtactagtgccatgagcagcggaactgtgactcaggataggaattctctccaagacaataagagcacagttgtaagctggcgagaacgtggtgcctcagatgctcgccgctacaatctggattcaatgccagagaatgacagctactcctctgcagctgaggatttctgtgaattatgcgaaacctcaggtcatgatgttctacattgcccgatgtttggccccaatggtaacagcagcaattctaaggatgagtcacctaaacagcaacgaacaggaaaagacgttgtcatggagggacttaaattatcacccaaaccttctcaagaagaatacaaaccggcgccgttagcgccagctaagaagtcgcctgatgcgtcgcctatcaagactgttcccaaccttatggaaccaggacctgccccaggaaaggaaagtggagtaatcaacatggataaatggtgcggtgtatgtgaaagagatggacatgacagtattgattgtccttttgaagatgctttttag

SEQ ID NO: 196 - RNA, 2892 nt, Botrytis cinerea betaendornavirus 1
  source 1..2892: mol_type = transcribed RNA
atgcctggcctcgttcgcaaactccttatctttgccgccatcgatgggttgattttgcaaccagcagcgccaaaaggccaacgccccgcccccgcaacgaagatcgcatacaaagataagcatatcgggccagtattgagtgatttgcaggatctggaggggtcgtctgcgaaaagtttcgaggcatttggtattgtcggtctcttgacggtttccaaaagctccttcctgatatcgattacgaaaagagagcaagtcgcacaaatacaagggaaacctatatatgttattactgaagtggctttgaccccattaagttccaagaacgaagcagagatctcgattgatagtacgaaagcggggttattgaagagtaatatcgaggggcagcatggcttggacgagagtgatagcgaggatgatgtcgttagcgatgaagtggaggacgatacagcagtagaagcacacaaaagaacgagtagcgtagctgaagatgtgatctcgaagaaggggggatatggaagatttgctcaaaaatggttctcgaagaaaggatgggccgtggaccagaagaagaacctggggatgagcgctgagccgtattccacagtggagcaagcttccaaggccaccgatgtaccagctacgatttcaggagtcactgaaggaaaatctgatatctcaattcccgataagggcaaggaaattgaggacattgaaactcctgaaaatattagcgacattgcagagagcatgctgccaaaattactacgaacatcgcagatattgtttggggcctctcggagttactacttttcttacgaccatgatatcacaagaagtttggcaaataagaggaatacaaattctgaattgccattgcacaaggaagttgatccactcttcttctggaatcggcatcttactttaccatttattgatgctggccagtcttctcttgccttgcctcttatgcagggctttgtaggacagcgtgcattttcaatggatagtaatccaccaaaccctgctataggttcagacactggaaagacttccgtgcagatgaaggatattacaacaagtagttcggatgagcaaatttacacagcacgtgctggtacagacaagtcgtatctattgacgttaatatctagaaggtcagtcaaacgtgccgggcttagatatttacgccggggtgtggatgaggacggcaatacagccaatggcgtggaaacagagcaaatcttatcggattctgcttggggcccttcgagtaagacatattcgttcgttcagatacgtggcagcattcccatattcttctcccagtcaccttactcttttaaacctgtacctcaagttcaccactctaccgaaacaaattatgaagctttcaagaagcattttgataatataagtgatcgctacggggccattcaagtggcttccttggtggagaagcatggaaacgaggcaatagtcggtggagagtacgagaaattgatgactctccttaatgtctcccgagctagcgagcttaggaaatccattgggtttgaatggtttgatttccatgctatttgcaaaggtatgaaatttgagaatgtcagcctgctcatggaaatactggacaagaagcttgactcgttttcgcacactgttgaaaccgatgggaaacttgtatcgaaacagaatggcgttttaaggactaactgtatggattgtctggatcgaacaaacgttgttcaaagtgcagtggcaaagcgagcacttgaaatgcagttaaagaatgagggactagatgtcactctacaaattgatcaaactcaacaatggttcaatactttgtgggccgacaatggtgacgccatttctaagcaatacgcttctacagcagcattgaagggagactttactcgtactaggaagcgggattataagggggccatcacagatatggggctttctatctccagattttatagcggcattgtaaatgactacttcagtcaagctgccattgatttcctgcttggaaatgtgagctatcttgtttttgaagacttcgaggcaaacatgatgagcggtgatcctggcgtttcgatgcaaaaaatgaggcaacaagccattgatgtttctcagaaactcgttgttgctgacgaccgtgaagaatttattggaggatggacatttctcactccgcaggtacccaatacgatcaaatctagtccttttgaggaatccgtcctcctattgacagatgctgcattgtatatgtgcaattttgattggaatatcgagaaagtatcatctttcgtgagagtggacttgaaccaggtgaacggcatcaagtttggaacatacatcacgagtactttgtcacaagcccaggcagatgagaagaggaatgtgggctttgtaataacttataaggctggttcaaacgacattattcgcgtgaacacgagatctatggctacggaatttccttcttcgaaactctctctcgaagacaaaacatccacgcccgcttctacatctaccaccaactctgtcgtcgccccaattgccgccgggtttgcaaacctaatctcaggtttacaaaatcaaagtatagcggaacctaaagatctcgtgaaggttctcgcattcaaggctctaccctccagatctgcggtatcagatgaaggagttagtgaggccgagcaagtgaagagtgtctgtggagagattagaagaatggttgagattggaagtataagagaggctggagaggagagaaaggatattgtagaggagggtactatcattagtttggccgaggccaagaaaagcacgggactattcgatgtgctgggacatcaggtgaagaaactggtttgggcttaa

SEQ ID NO: 197 - RNA, 1608 nt, Botrytis cinerea betaendornavirus 1
  source 1..1608: mol_type = transcribed RNA
atgggattaccaccatgggagacaagtgagagccagacttttgccttaataacaggcgcaaacagcggcttgggttttgccattgcttctagattgattgacgaattcctgacttcatctgatactcctcctactaaacatttgattctcatcctttgcacgcgtacacctctgaagacacgattcacaatctcccgcctgcgtgctcatctacgaaaactggccgactactctgaattcgcaacttcacatcgagcgaaagctaagtctcagggaaatgtatatagatggcaggatacggtggctcgggttcattttcttggggttgaagttgacttgtgcgacttgaaaagtgtatatgctctcaccgataggcttgtcaatggaactgttggtagcccagatgctactacaatggatggtctccgattacctgatggctctcctggtaccgccacttattccgcagatgttaaacaagacagatgggcattgagtcagaaggaagggtctgaaggcgagctgagatcttggggatggggattgagcggaattaggataccaaggctggatgttgtagtcttgaatgcagggataggaggatggtcaggaatcgattggccaaaggctatatggactgtcataacagatatgacggaagctgtaacatggccaacttacaagcttgcagaaattggagttatcaccaaacctcaactatcctctgcctcttcaaaacaagccaaaccctccgacgatgaagctgcgcaacctttactcgacggtgaatctccggaagaaccacctcttggagcaacattctgttctaacgttttcggacattacgttctcgcacacgagctgatgcctttactatcgcgaactgcttctccttcggccactaccagcggaagaataatatgggtgtctagtatcgaggcacaggcacaacattttgatgaagatgatttacaaggtttggaaagtcgcacgccatacgaaagctccaaacgtcttacagatgttctcgtcctttcaagaaaattacgagcagcaggccaagcctcctcttcatggttcgattgttctgacgttcgcgtggagaactctaaatcggaggaagaaccagcagcaaaattgataagaccgaaaatgtacgtggttcaacctggaatttttgtttcggagatcatgcccttgaattttgtgttggtatttatctacagattgatcatctaccttgtaagatggatgggaagccaatggcataccatcaagccttacactgctgctgtagcaccagtctgggtagcattatctcccgacgatgttctagataacatggacggggcagcttcgaaatggggatcagctacagatgctagtgggaaagaacgcgttatacgaaccgaagttcctggttggggatgggaaggcaaaactccaaagacaattgatactggagagagaagaaaggggaggcaaagaaatgcggaaccattgacgagggaagcgagagaggattttgaggtcttgggtgttaagtgttggacggagatggagaatttgaggaaagaatgggagggacttttgaaggttaaaaaatga

SEQ ID NO: 198 - RNA, 2604 nt, Botrytis cinerea betaendornavirus 1
  source 1..2604: mol_type = transcribed RNA
atggtcttgttggtatcaaaaagagggtgtcgagtatggcatcgatacttgacacaagttacatggccttgtctggctaagcctagtcaattgaatgcgttcattcgttatagttcacagcagactgaaagtcatgatacgttaacagagacaactcgaaatattggcatcatagctcatatcgatgcaggcaaaactacaactactgagcgtatgctctattacagtggctatactcgacgcataggagacgttgatgatggctccaccgtcacagacttcctccccgccgagagggctagagggattactattcagtcggcagccgttacgatgcactggccccctgtgactgagaaagcagcatcctcgaaagcgtctgacccatctcgatcacttatatcgcacactcttaacctgattgatactcccgggcacgcggattttacgtttgaagtgcttcgttctttgagaatccttgatggtgccgtatgtattcttgatggtgtggcaggagtagaagctcaaacagaaaaagtatggaaacaggcaaataattatagcattcccaggatcgctttcgtcaataagcttgatcgtgaaggggctgccttcgcgagaacagtaaaagagattgcttcgaggctccggggctggcctgcggtgtgtcaaattccatggtgggaaggtgggaaaggaaagtttacgggagtcggtgatgcagtcaatctttgtgcgctgaaatgggaagaaggtggggatggcaaatcaatccaacattttaccctcgatcagctgaggaaagataatcctgaattttccgaagaaatcatcaaggcgcgagctgcgctcgtagaggcattatgcgaatttgatgatgggctccttgaaacctggctagaatgtaatgatgacagtctgcttatatcatcagcggacattacaaagagtttgcgaaaatgcgtactcgacggttcgggtaaactcatacctgtctttgctggggccagttttcgaaatattggcgttcaaccactccttgatgccatcaataatcttctacccaaccctaccgaaaggcctgaaccagaagttcgacttggcaatgttcatggcagtttatcccaactcctagatggaaagctggaccttagcgcagcgcaaccaagacatctctccaagaaatccaatgcgcgtacgtctctcatttctcaggtcgaagcttgtgcccttgctttcaaggtagtcaatgatgctcgacgcggcgtgttagtctacatcagagtttattccggtacagtcaagcggaacactactttatggaatacgaatcttcatgtttcagaaagagcacaaaggctgttacagatgtacgcatctgacgcggtagagatacaaagcattccctccggtcagattggcgttattgcgggcttgaagcacgctcgtacaggcgatactctattgtcatatacaggtgctcatccaaaaaatggcccgccaccacctttgaatactcttcaactgagaccaattaatgttcctccgccagtattttttgccgctatagaacctcacagtctaagcgaagaaaaaaatgttgccgacatattgcagctcttattgagggaagacccaagtctccatgttaatattgatgaagaatctgggcaaatgcagttgagtggtatgggtgagctgcatcttgaaatcgcaaaagatcgactcgtaaacgatttcaaagccaaggcaaccatgggcaatatcgaaattgggtaccgagaatgcgtcctgtctccaacattacctcacaaatatatatttgatcgtgaagttgctggcaaaaaaggaaaagcaagctgcgaagctagtatcagtccagacgcgcagccgttagaagattctgaccacactatgaacattgatggaaatacaatcacaatccgtatcccaaaaccttctaacaatgatggggttgatggaactatgacactcccctccgatatgaccctcagcgaagttcatacagcattgatcaatggggctgttgctggtctagcccgtggtccgcgtcgtgcattcccacttcattctgcgcatgtgctattgaagtttgataccgttgaggatgtctttggttccgacactacttctgccgcattgtcttctgcgtcaagaaatgccgtacaagctgctctcaaagaagcatttcaagcgaactccatcggactgatggaaccagtcatgaatgtggttattagttgcgacgaatcatccctcggtgcaattgtgcacgatctatcatcagctcgtggtggccatgtcttatcacttgagaatgatagtgacgtagaggatacagaaaatgagctggcgccagttgatgtttcaagagtctatactcctccagatccattcgcgtcaggaaccagtactgattcatcgggtcctggccagcagcgtcaaatcaccgctagagtaccattgaaagagatggttggatatttgaagcatttgaggagcatgactggcggtagaggaacattcgtcatgagcgttgataggtttgaaagactttctgggccaagagaaaaggctttgtag

SEQ ID NO: 199 - RNA, 2793 nt, Botrytis cinerea betaendornavirus 1
  source 1..2793: mol_type = transcribed RNA
atgtcctataatcgattagatccggcgggccaaggccaagacgattattacaatatgaataatagacatcaatcgccgcaccctcaagggtaccaactagaagatgcgccatatggcagaccaaatactacttcacccggtcctggaatgcacaatctagagatacctatgggtcctggggcacatagaattggaacgccgagtgatcaattgcaagctcaaccatcttattcggtcgaacatttagatcaaaatcaataccatcagcgcatgcccctcaatcccagtcaaagctacgactcggaatattctttagatcctaacgcgcatcacgatgcttactaccaacctccataccaaccctctcctcatgaagaacaccctctacagaactatgccccagggcaagacccctacgcttacaatgatgatgatgaccatcaaccaattctacaatcgcatgaaccttatgggccagatccgcactcagctagtggcactgattacaaaggtggttatgacgggacggtacaatctccatcagcgacacctgtacctgcgttaagaagatacaagacggtcaaggaagtccaactgttcaatggaaatctcgtactcgattgtccgattcctcccaagcttttaaatcaagtcaatcatgcaccaccgccggagagagatgagttcacacatatgagatattcagccgcaacatgcgacccctctgagttttttgaggagcgctttacattgcgacagaaactcttcgcaaagcctcgacacacagaactcttcatcgttgtcacaatgtataatgaagatgatgtattgtttgctagaacaatgcacggagtattcaagaacattgaatttatgtgcactcgtaaagacagtaaaacatggggcaaggatgcttggaagaagatcgtagtgtgtgtggtcagtgatggacgtgccaaaatcaatccaagaacaagggctgttttggctggtttgggggtttatcaggacggaattgcgaagcaacaagtcaatggcaaggacgtgacagcacacatctatgaatatacgactcaagtcggaatttctttgaaaaaggatattgttacactcacaccaaaacagcaacccgttcaattgcttttctgtttgaaggaaaagaatcagaaaaagatcaactctcacagatggttcttccaagcctttggtagagtacttgatcccaacatttgtgtactcctcgatgctggtacaaaaccaggaaaggactcaatttatcatctatggaaagctttcgatttggaaccacattgtgcaggagcttgtggtgagatcaaagctatgttgggcccaggaggaaagaatttggtcaatccattggttgctacccagaatttcgagtacaagatgagtaatattctggacaaacctcttgaatcggcatttgggttcatttcggtgttgccaggtgctttttctgcatatcgatatgtcgcgttacaaaacgataaaactggaaatggaccactggagaagtactttgcaggagagaagatgcatggagcaaacgcgggtatttttactgccaacatgtaccttgccgaagatcgtattttgtgtttcgaactggtatcaaagagaaattgtcactggatcttacaatacgtcaagtctgctactggagaaaccgatgtaccagatacaatggcggaacttattttgcaacgtcgaagatggcttaacggaagtttcttcgctgctatctatgctcttgctcatttttatcaaattttccgaagtgatcacagctttttacgaaaaatcatgtttttgattgaattcacatatcaaactattaacatgatcttcgcttggttcgctcttggtaatttcttcttggtttttcacatcttgactacatctctcggaagttctgacttactgggtaacgttggtgtaattcttggtgttgttttcgaatggctttacttgtttacgcttttgacctgttttattctggcgctgggaaatcgacctcaaggaacgaacaaagtttatatgtctatggtttatttctggatcattatcatgatatacctaatgtttgcttcgattttcatcacggttaaatcaatccaaactcaacttgctaaagacgaattcaactggacggatattatcaagaatcagatcttctatactctgatcatttctctcgcctcaacttatctactctggttcatttcttcctttttattcttcgacccatggcacatgtttacatctttccttcaataccttcttctcactccaacatatatcaatattctcaacgtttacgctttctgtaacactcacgatattacatggggtacaaaaggagatgacaaagccgagaaacttccatccgctgtgctcaaagctggtggtaaagtcgacgtcaatattcccaccgacgacggtgatctcaacgcccaatatgaatcggaaatgcgcaagattcagatcaaagctccacctgagaaacgtgaattctcggcagaagagaagcaagaggactattataaatggttcagatcttcggtagtgttgttctggttggtttgtaattttgcactcacgagtgcggtgcttagtacggcgggcttggaaaaatttggtaccggtactgatgatacgacgaagagtacgatttacatggctgtggttttatggagtgtggcaggattgagttgtttcaagtttattggtgcgatgtggtttttgattgttaggatgtttagaggtgtttag

SEQ ID NO: 200 - DNA, 766 bp, synthetic construct
  source 1..766: mol_type = other DNA
ggactagttaatacgactcactatagggcgaattgggtaccgggcattacgtttcttaattgctgtatactcttcttatgatacgttatcagatttttcaaggtaatctatagtctgcactttcgacgaaagagtaagaacttcgaacaaaaaagcgacaaggagctcatcatggtatgttctagcgcttgcaccatcccatttaactgtaagaagaattgcacggtcccaattgctcgagagatttctcttttacctttttttactatttttcactctcccataacctcctatattgactgatctgtaataaccacgatattattggaataaataggggcttgaaatttggaaaaaaaaaaaaaactgaaatattttcgtgataagtgatagtgatattcttcttttatttgctactgttactaagtctcatgtactaacatcgattgcttcattctttttgttgctatattatatgtttagagtgatgagctccttgtcgcttttttgttcgaagttcttactctttcgtcgaaagtgcagactatagattaccttgaaaaatctgataacgtatcataagaagagtatacagcaattaagaaacgtaatgcccggtacccaattcgcccggccggcatggtcccagcctcctcgctggcgccggctgggcaacattccgaggggaccgtcccctcggtaatggcgaatgggaccctagcatatccatgatatctgttagtttttttcctgaaaggtctagagc

SEQ ID NO: 201 - DNA, 942 bp, synthetic construct
  source 1..942: mol_type = other DNA
ggactagttaatacgactcactatagggcgaattgggtaccgggcattacgtttcttaattgctgtatactcttcttatgatacgttatcagatttttcaaggtaatcttgatgagctccttgtcgcttttttgttcgaagttcttactctttcgtcgaaagtgcagactattctcagatctgccggtctcccggccggcatggtcccagcctcctcgctggcgccggctgggcaacattccgaggggaccgtcccctcggtaatggcgaatgggaccctagcatatccatgatatctgttagtttttttcctgaaagaatgttctagcgcttgcaccatcccatttaactgtaagaagaattgcacggtcccaattgctcgagagatttctcttttacctttttttactatttttcactctcccataacctcctatattgactgatctgtaataaccacgatattattggaataaataggggcttgaaatttggaaaaaaaaaaaaaactgaaatattttcgtgataagtgatagtgatattcttcttttatttgctactgttactaagtctcatgtactaacatcgattgcttcattctttttgttgctatattatatgtttaatacgactcactatagggagaccggcagatctgagaatagtctgcactttcgacgaaagagtaagaacttcgaacaaaaaagcgacaaggagctcatcaagattaccttgaaaaatctgataacgtatcataagaagagtatacagcaattaagaaacgtaatgcccggtacccaattcgcccggccggcatggtcccagcctcctcgctggcgccggctgggcaacattccgaggggaccgtcccctcggtaatggcgaatgggaccctagcatatccatgatatctgttagtttttttcctgaaaggtctagagc

SEQ ID NO: 202 - DNA, 760 bp, synthetic construct
  source 1..760: mol_type = other DNA
cccaagcttggggtgcttcggatgctgatgagtccgtgaggacgaaacagggcaacctgtccatccggtatcccaccgggcattacgtttcttaattgctgtatactcttcttatgatacgttatcagatttttcaaggtaatctatagtctgcactttcgacgaaagagtaagaacttcgaacaaaaaagcgacaaggagctcatcatggtatgttctagcgcttgcaccatcccatttaactgtaagaagaattgcacggtcccaattgctcgagagatttctcttttacctttttttactatttttcactctcccataacctcctatattgactgatctgtaataaccacgatattattggaataaataggggcttgaaatttggaaaaaaaaaaaaaactgaaatattttcgtgataagtgatagtgatattcttcttttatttgctactgttactaagtctcatgtactaacatcgattgcttcattctttttgttgctatattatatgtttagagtgatgagctccttgtcgcttttttgttcgaagttcttactctttcgtcgaaagtgcagactatagattaccttgaaaaatctgataacgtatcataagaagagtatacagcaattaagaaacgtaatgcccggtgggataccggatgggccggcatggtcccagcctcctcgctggcgccggctgggcaacattccgaggggaccgtcccctcggtaatggcgaatgggactctagagc

SEQ ID NO: 203 - DNA, 900 bp, synthetic construct
  source 1..900: mol_type = other DNA
ggactagttgaagtttttctcggcgagaaatacgtagttaaggcagagcgacagagagggcaaaagaaaataaaagtaagattttagtttgtaatgggagggggggtttagtcatggagtacaagtgtgaggaaaagtagttgggaggtacttcatgcgaaatgggtaccgggcattacgtttcttaattgctgtatactcttcttatgatacgttatcagatttttcaaggtaatctatagtctgcactttcgacgaaagagtaagaacttcgaacaaaaaagcgacaaggagctcatcatggtatgttctagcgcttgcaccatcccatttaactgtaagaagaattgcacggtcccaattgctcgagagatttctcttttacctttttttactatttttcactctcccataacctcctatattgactgatctgtaataaccacgatattattggaataaataggggcttgaaatttggaaaaaaaaaaaaaactgaaatattttcgtgataagtgatagtgatattcttcttttatttgctactgttactaagtctcatgtactaacatcgattgcttcattctttttgttgctatattatatgtttagagtgatgagctccttgtcgcttttttgttcgaagttcttactctttcgtcgaaagtgcagactatagattaccttgaaaaatctgataacgtatcataagaagagtatacagcaattaagaaacgtaatgcccggtacccatttcgcatggccggcatggtcccagcctcctcgctggcgccggctgggcaacattccgaggggaccgtcccctcggtaatggcgaatgggacctctataaattttatttgtcttaagaattctatgatccgggtaaaaatctagagc

SEQ ID NO: 204 - DNA, 1210 bp, synthetic construct
  source 1..1210: mol_type = other DNA
ggactagttgaagtttttctcggcgagaaatacgtagttaaggcagagcgacagagagggcaaaagaaaataaaagtaagattttagtttgtaatgggagggggggtttagtcatggagtacaagtgtgaggaaaagtagttgggaggtacttcatgcgaaatgggtaccgggcattacgtttcttaattgctgtatactcttcttatgatacgttatcagatttttcaaggtaatcttgatgagctccttgtcgcttttttgttcgaagttcttactctttcgtcgaaagtgcagactatgggagaccggcagtttcgcatggccggcatggtcccagcctcctcgctggcgccggctgggcaacattccgaggggaccgtcccctcggtaatggcgaatgggacctctataaattttatttgtcttaagaattctatgatccgggtaaaaaatgttctagcgcttgcaccatcccatttaactgtaagaagaattgcacggtcccaattgctcgagagatttctcttttacctttttttactatttttcactctcccataacctcctatattgactgatctgtaataaccacgatattattggaataaataggggcttgaaatttggaaaaaaaaaaaaaactgaaatattttcgtgataagtgatagtgatattcttcttttatttgctactgttactaagtctcatgtactaacatcgattgcttcattctttttgttgctatattatatgtttgaagtttttctcggcgagaaatacgtagttaaggcagagcgacagagagggcaaaagaaaataaaagtaagattttagtttgtaatgggagggggggtttagtcatggagtacaagtgtgaggaaaagtagttgggaggtacttcatgcgaaactgccggtctcccatagtctgcactttcgacgaaagagtaagaacttcgaacaaaaaagcgacaaggagctcatcaagattaccttgaaaaatctgataacgtatcataagaagagtatacagcaattaagaaacgtaatgcccggtacccatttcgcatggccggcatggtcccagcctcctcgctggcgccggctgggcaacattccgaggggaccgtcccctcggtaatggcgaatgggacctctataaattttatttgtcttaagaattctatgatccgggtaaaaatctagagc